European Patent Application EP 4 729 542 A1, published April 22, 2026. Title: ANTIGEN-BINDING POLYPEPTIDES AGAINST CD229. Applicant: Universitätsklinikum Hamburg-Eppendorf. The sequence listing filed with the application follows.

SEQUENCE LISTING (143 sequences)

SEQ ID NO: 1 - protein, 4 aa, Vicugna pacos
  source 1..4: note = only amino acids 1-3 (I-F-I) represent the CDR, while the amino acid M does not belong to the CDR
IFIM

SEQ ID NO: 2 - protein, 5 aa, Vicugna pacos
SSRGS

SEQ ID NO: 3 - protein, 12 aa, Vicugna pacos
GAETILGPPGAY

SEQ ID NO: 4 - protein, 4 aa, Vicugna pacos
  source 1..4: note = only amino acids 1-3 (I-F-I) represent the CDR, while the amino acid M does not belong to the CDR
IFIM

SEQ ID NO: 5 - protein, 5 aa, Vicugna pacos
SSRGS

SEQ ID NO: 6 - protein, 12 aa, Vicugna pacos
GAQTLLGPPGAY

SEQ ID NO: 7 - protein, 6 aa, Vicugna pacos
TFSNYY

SEQ ID NO: 8 - protein, 6 aa, Vicugna pacos
SVIWDA

SEQ ID NO: 9 - protein, 18 aa, Vicugna pacos
GRGPMFTSRWHDELWYES

SEQ ID NO: 10 - protein, 6 aa, Vicugna pacos
PFDAYN

SEQ ID NO: 11 - protein, 6 aa, Vicugna pacos
RWNGLS

SEQ ID NO: 12 - protein, 18 aa, Vicugna pacos
TLNWLHAHEAMGQIKYNH

SEQ ID NO: 13 - protein, 6 aa, Vicugna pacos
TLSRNV

SEQ ID NO: 14 - protein, 6 aa, Vicugna pacos
SWSGDR

SEQ ID NO: 15 - protein, 15 aa, Vicugna pacos
TREMLMGTPTRKYDY

SEQ ID NO: 16 - protein, 6 aa, Vicugna pacos
SLDTRA

SEQ ID NO: 17 - protein, 6 aa, Vicugna pacos
SSSDGS

SEQ ID NO: 18 - protein, 14 aa, Vicugna pacos
PYGSTCQTYYGMDY

SEQ ID NO: 19 - protein, 6 aa, Vicugna pacos
TLDTRA

SEQ ID NO: 20 - protein, 6 aa, Vicugna pacos
SSTDSS

SEQ ID NO: 21 - protein, 14 aa, Vicugna pacos
PYGSTCRTYYGMDY

SEQ ID NO: 22 - protein, 6 aa, Vicugna pacos
TLDTRA

SEQ ID NO: 23 - protein, 6 aa, Vicugna pacos
SSSDGD

SEQ ID NO: 24 - protein, 14 aa, Vicugna pacos
PFGSTCRTYYGMDY

SEQ ID NO: 25 - protein, 6 aa, Vicugna pacos
TLDTRA

SEQ ID NO: 26 - protein, 6 aa, Vicugna pacos
SSSDGR

SEQ ID NO: 27 - protein, 14 aa, Vicugna pacos
PFGTTCRTYYGMDY

SEQ ID NO: 28 - protein, 6 aa, Vicugna pacos
AISSYS

SEQ ID NO: 29 - protein, 6 aa, Vicugna pacos
SRIGGR

SEQ ID NO: 30 - protein, 14 aa, Vicugna pacos
STFNVADVTSMYDY

SEQ ID NO: 31 - protein, 6 aa, Vicugna pacos
TLRYYA

SEQ ID NO: 32 - protein, 6 aa, Vicugna pacos
SHNGGN

SEQ ID NO: 33 - protein, 14 aa, Vicugna pacos
KCAFGTIPTSWYDS

SEQ ID NO: 34 - protein, 6 aa, Vicugna pacos
TLDNYA

SEQ ID NO: 35 - protein, 6 aa, Vicugna pacos
SSVDGS

SEQ ID NO: 36 - protein, 15 aa, Vicugna pacos
SPYGRSCATYYGMDY

SEQ ID NO: 37 - protein, 6 aa, Vicugna pacos
TFNLFA

SEQ ID NO: 38 - protein, 6 aa, Vicugna pacos
TKSGRS

SEQ ID NO: 39 - protein, 13 aa, Vicugna pacos
GDSISSTSASYNA

SEQ ID NO: 40 - protein, 6 aa, Vicugna pacos
TDNLFA

SEQ ID NO: 41 - protein, 6 aa, Vicugna pacos
TKSGRS

SEQ ID NO: 42 - protein, 13 aa, Vicugna pacos
GDSISSTSASYNA

SEQ ID NO: 43 - protein, 8 aa, Vicugna pacos
GWFVSMHD

SEQ ID NO: 44 - protein, 5 aa, Vicugna pacos
ERHGN

SEQ ID NO: 45 - protein, 7 aa, Vicugna pacos
HLGARDY

SEQ ID NO: 46 - protein, 6 aa, Vicugna pacos
IFSRND

SEQ ID NO: 47 - protein, 5 aa, Vicugna pacos
TVIGN

SEQ ID NO: 48 - protein, 7 aa, Vicugna pacos
GTLTYDY

SEQ ID NO: 49 - protein, 6 aa, Vicugna pacos
IFSRND

SEQ ID NO: 50 - protein, 7 aa, Vicugna pacos
GTLTYDY

SEQ ID NO: 51 - protein, 7 aa, Vicugna pacos
GTLTYDY

SEQ ID NO: 52 - protein, 6 aa, Vicugna pacos
ISSIVD

SEQ ID NO: 53 - protein, 5 aa, Vicugna pacos
PGTGV

SEQ ID NO: 54 - protein, 11 aa, Vicugna pacos
SEWRGARVFGS

SEQ ID NO: 55 - protein, 6 aa, Vicugna pacos
ISSIVH

SEQ ID NO: 56 - protein, 5 aa, Vicugna pacos
PGTGS

SEQ ID NO: 57 - protein, 11 aa, Vicugna pacos
SEWRGARVFGS

SEQ ID NO: 58 - protein, 6 aa, Vicugna pacos
TNTIKH

SEQ ID NO: 59 - protein, 5 aa, Vicugna pacos
DSDGD

SEQ ID NO: 60 - protein, 11 aa, Vicugna pacos
ALATSSGLYYY

SEQ ID NO: 61 - protein, 6 aa, Vicugna pacos
TNTIKH

SEQ ID NO: 62 - protein, 5 aa, Vicugna pacos
DSDGD

SEQ ID NO: 63 - protein, 11 aa, Vicugna pacos
ALATSSGLYYY

SEQ ID NO: 64 - protein, 6 aa, Vicugna pacos
TFSLYY

SEQ ID NO: 65 - protein, 6 aa, Vicugna pacos
RWSDMT

SEQ ID NO: 66 - protein, 9 aa, Vicugna pacos
AAASGRYDY

SEQ ID NO: 67 - protein, 6 aa, Vicugna pacos
TFSLYY

SEQ ID NO: 68 - protein, 6 aa, Vicugna pacos
RWSDGT

SEQ ID NO: 69 - protein, 9 aa, Vicugna pacos
AAASGRYDY

SEQ ID NO: 70 - protein, 6 aa, Vicugna pacos
TFSRNV

SEQ ID NO: 71 - protein, 6 aa, Vicugna pacos
SEISGT

SEQ ID NO: 72 - protein, 14 aa, Vicugna pacos
GSMVYAIMPEYYDV

SEQ ID NO: 73 - protein, 6 aa, Vicugna pacos
TFSRNV

SEQ ID NO: 74 - protein, 6 aa, Vicugna pacos
SEISGT

SEQ ID NO: 75 - protein, 14 aa, Vicugna pacos
GSMVFATMPEYYDY

SEQ ID NO: 76 - protein, 6 aa, Vicugna pacos
TFSRNV

SEQ ID NO: 77 - protein, 6 aa, Vicugna pacos
SEISGT

SEQ ID NO: 78 - protein, 14 aa, Vicugna pacos
GSMVYAIMPEYYDV

SEQ ID NO: 79 - protein, 6 aa, Vicugna pacos
TFSRNV

SEQ ID NO: 80 - protein, 6 aa, Vicugna pacos
SEISGT

SEQ ID NO: 81 - protein, 14 aa, Vicugna pacos
GSMVYAIMPEYYDV

SEQ ID NO: 82 - protein, 4 aa, Vicugna pacos
  source 1..4: note = only amino acids 1-3 (T-F-G) represent the CDR, while the amino acid I does not belong to the CDR
TFGI

SEQ ID NO: 83 - protein, 6 aa, Vicugna pacos
QWSGSG

SEQ ID NO: 84 - protein, 13 aa, Vicugna pacos
GRTYYSQQDSYDS

SEQ ID NO: 85 - protein, 6 aa, Vicugna pacos
AFSRSY

SEQ ID NO: 86 - protein, 5 aa, Vicugna pacos
QTNDY

SEQ ID NO: 87 - protein, 13 aa, Vicugna pacos
EQSLMTDMEEFEF

SEQ ID NO: 88 - protein, 5 aa, Vicugna pacos
ISSYH

SEQ ID NO: 89 - protein, 6 aa, Vicugna pacos
DSSGHS

SEQ ID NO: 90 - protein, 13 aa, Vicugna pacos
GRWPTVKAAFVDS

SEQ ID NO: 91 - protein, 5 aa, Vicugna pacos
ISSYH

SEQ ID NO: 92 - protein, 6 aa, Vicugna pacos
DSSGHS

SEQ ID NO: 93 - protein, 13 aa, Vicugna pacos
GRWPTVKAAFVES

SEQ ID NO: 94 - protein, 6 aa, Vicugna pacos
TVSSYF

SEQ ID NO: 95 - protein, 6 aa, Vicugna pacos
NWTGDN

SEQ ID NO: 96 - protein, 13 aa, Vicugna pacos
GRWPTVRPESIDS

SEQ ID NO: 97 - protein, 6 aa, Vicugna pacos
TDSSYF

SEQ ID NO: 98 - protein, 6 aa, Vicugna pacos
NWASDN

SEQ ID NO: 99 - protein, 13 aa, Vicugna pacos
GRWPTVRPESIDS

SEQ ID NO: 100 - protein, 6 aa, Vicugna pacos
TDSSYF

SEQ ID NO: 101 - protein, 6 aa, Vicugna pacos
NWDGDN

SEQ ID NO: 102 - protein, 13 aa, Vicugna pacos
GRWPTVRPGSVTS

SEQ ID NO: 103 - protein, 117 aa, Vicugna pacos
QVKLQESGGGLVQPGGSLRLSCAASGNIFIMGWYRQAVGQQRELVALISSRGSLNYGAAVLGRFTISRDNAKKMVYLQMDRLKPEDTAHYYCNAGAETILGPPGAYWGQGTQVTVSS

SEQ ID NO: 104 - protein, 117 aa, Vicugna pacos
QVKLQESGGGSVQPGGSLRLSCVASGSIFIMGWYRQAAGQQRELVALISSRGSLNYGEAVLGRFTISRDNAKKMVYLQMDRLKPEDTAHYYCNAGAQTLLGPPGAYWGQGTQVTVSA

SEQ ID NO: 105 - protein, 127 aa, Vicugna pacos
QVKLQESGGGLAQAGGSLRLSCAASGGTFSNYYMGWFRQAPGKQREPIAAVSVIWDATYHAPSALGRFTISRDNAKNTVSLQMNSLKPEDTAVYYCAAGRGPMFTSRWHDELWYESWGQGTQVTVSS

SEQ ID NO: 106 - protein, 127 aa, Vicugna pacos
DVQLQASGGGLVKVGDSLTLSCEFSGGPFDAYNFGWFRQAPGREREFVGAIRWNGLSTDYADSMKGRFAISRDDAKNAVFLQMYDVRPEDTAVYFCAATLNWLHAHEAMGQIKYNHWGQGTQVTVSS

SEQ ID NO: 107 - protein, 124 aa, Vicugna pacos
QVKLQESGGGVVQAGGSLRLSCAASGGTLSRNVVGWFRRAPGKEREFVVASSWSGDRPIYADSVAGRFIVSRDNAKNTVYLQMNSLKPEDTAVYYCAATREMLMGTPTRKYDYWGQGTQVTVSS

SEQ ID NO: 108 - protein, 123 aa, Vicugna pacos
QVQLQESGGGLVQPGGSLRLSCAASGFSLDTRAIGWFRQVPGKEREEVSCISSSDGSTRYADSVKGRFTISRDLSKNTVYLQMNSLKSEDTAVYYCGTPYGSTCQTYYGMDYWGKGTLVTVSS

SEQ ID NO: 109 - protein, 123 aa, Vicugna pacos
QVQLQESGGGLVQPGGSLRLSCAASGFTLDTRAIGWFRQAPGKEREEVSCISSTDSSTRYADSVKGRFTISRDLSKNTVYLQMNSLKSEDTAVYYCGTPYGSTCRTYYGMDYWGKGTLVTVSS

SEQ ID NO: 110 - protein, 123 aa, Vicugna pacos
QVQLQESGGGLVQPGGSLKLSCAASGFTLDTRAIGWFRQAPGKEREEVSCISSSDGDTRYADSVKGRFTISRDLSKNTVYLQMNSLKSEDTAVYYCGTPFGSTCRTYYGMDYWGKGTLVTVSS

SEQ ID NO: 111 - protein, 123 aa, Vicugna pacos
DVQLQASGGGLVQPGGSLRLSCAASGFTLDTRAIGWFRQAPGKEREEVSCISSSDGRTRYADSVKGRFTISRDLSKNTVYLQMNSLKSEDTAVYYCGTPFGTTCRTYYGMDYWGKGTLVTVST

SEQ ID NO: 112 - protein, 123 aa, Vicugna pacos
QVKLQESGGGLVQAGDSLRLSCAASGRAISSYSMGWFRQAPGKEREFVTTISRIGGRTFYADFVKGRFTISRDNARNTGYLQMDSLKPEDTAVYYCGVSTFNVADVTSMYDYWGQGTQVTVSS

SEQ ID NO: 113 - protein, 123 aa, Vicugna pacos
DVQLQASGGGLVQPGGSLRVSCAASGSTLRYYAIGWFRQAPGKEREGISCISHNGGNTNYADSVKGRFTVSRDNAKNTVYLQMTSLKLEDTAVYYCAPKCAFGTIPTSWYDSWGQGTQVTVSS

SEQ ID NO: 114 - protein, 123 aa, Vicugna pacos
QVQLQESGGGLVQPGGSLRLSCAVSGRTLDNYAIGWFRQAPGKEREWVSCISSVDGSTHYADSVKGRFTISRDNAKNTVYLQMDSLKPEDTAVYYCASPYGRSCATYYGMDYWGKGTLVTVSS

SEQ ID NO: 115 - protein, 122 aa, Vicugna pacos
QVQLQESGGGLVQAGGSLRLSCAASGRTFNLFAITWFRQAPGKEREFVAAITKSGRSVNYADSVNGRFTVSRNNVETTFYLQMDYLKPEDTAIYYCAAGDSISSTSASYNAWGRGTQVTVSS

SEQ ID NO: 116 - protein, 122 aa, Vicugna pacos
QVQLQESGGGLVQAGGSLRLSCAASGRTDNLFALTWFRQAPGKEREFVAAITKSGRSVNYADSVNGRFTVSRNNVETTFYLQMDHLKPEDTAIYYCAAGDSISSTSASYNAWGRGTQVTVSS

SEQ ID NO: 117 - protein, 117 aa, Vicugna pacos
QVKLQESGGGLVQPGGSLRLSCAGSGSGWFVSMHDMGWYRRAPGKARELVAAIERHGNIMYRDFVKGRFTISRDNAKNTVDLQMNSLEPEDTAVYYCNAHLGARDYWGQGTQVTVSA

SEQ ID NO: 118 - protein, 115 aa, Vicugna pacos
DVQLQESGGGLVQAGGSLRLSCAASGIIFSRNDMAWYRQAPRKERELVAVITVIGNTNYADSVKGRFTISRDDSKNTVSLQMNSLKPEDTAVYYCNVGTLTYDYWGQGTQVTVSS

SEQ ID NO: 119 - protein, 115 aa, Vicugna pacos
DVQLQASGGGLVQAGGSLRLSCAASGIIFSRNDMAWYRQAPRKERELVAVITVIGNTNYADSVKGRFTISRDDSKNTVSLQMNSLKPEDTAVYYCNVGTLTYDYWGQGTQVTVSS

SEQ ID NO: 120 - protein, 119 aa, Vicugna pacos
DVQLQASGGGLVQPGGSLRLSCAASGSISSIVDMGWYRQGPGKERELVATAPGTGVTHVADSVKGRFTISRDNAKNAVSLQMNNLKPEDTAVYYCYASEWRGARVFGSWGQGTQVTVSS

SEQ ID NO: 121 - protein, 119 aa, Vicugna pacos
QVQLQESGGGLVQAGGSLRLSCAASGTISSIVHMGWYRQGPGKERELVATAPGTGSTNYADSVKGRFTISRDNAKNTVSLQMNNLKPEDTAVYYCYASEWRGARVFGSWGQGTQVTVSS

SEQ ID NO: 122 - protein, 118 aa, Vicugna pacos
QVKLQESGGGSVQAGGSLRLSCAASGNTNTIKHIGWYQALGQQRELVAIIDSDGDTTYGDDVKGRFTISRDNAKNTVHLQMNSLQPEDTAVYRCAVALATSSGLYYYWGQGTQVTVSS

SEQ ID NO: 123 - protein, 118 aa, Vicugna pacos
QVQLQESWGGSVQAGGSLTLSCQASGNTNTIKHIGWYQALGQQRELVAIIDSDGDTTYGDDVKGRFTISRDNAKNTVHLQMNSLQPEDTAVYRCAVALATSSGLYYYWGQGTQVFVSS

SEQ ID NO: 124 - protein, 118 aa, Vicugna pacos
DVQLQASGGGLVQAGDSLRLSCAASGRTFSLYYMGWFRQAPGKEREFVGTIRWSDMTVHYSDSVKGRFTVSTDNPKNAVYLQMTSLKAEDTAVYYCAAAAASGRYDYWGQGTQVTVSS

SEQ ID NO: 125 - protein, 118 aa, Vicugna pacos
DVQLQESGGGSVQAGDSLRLSCAASGHTFSLYYMGWFRQAPGKEREFVGTIRWSDGTVHYSDSVKGRFSVSTDNPKNAVYLQMTSLKAEDTAVYYCAAAAASGRYDYWGQGTQVTVSS

SEQ ID NO: 126 - protein, 123 aa, Vicugna pacos
DVQLQASGGGLVQAGGSLRLSCAPSGRTFSRNVVGWFRQAPGREREFVAHISEISGTTHYADSVKGRFTISRINAENTVYLLMNSLKPEDTAIYYCAAGSMVYAIMPEYYDVWGQGIQVTVSS

SEQ ID NO: 127 - protein, 123 aa, Vicugna pacos
QVKLQESGGGLVQAGGSLRLSCAPSGRTFSRNVVGWFRQAPGREREFVAHISEISGTTHYADSVKGRFTISRINAENTVYLLMNNVKPEDTAIYYCAAGSMVFATMPEYYDYWGQGIQVTVSS

SEQ ID NO: 128 - protein, 123 aa, Vicugna pacos
QVKLQESGGGLVQAGGSLRLSCAPSGRTFSRNVVGWFRQAPGREREFVAHISEISGTTHYADSVKGRFTISRINAENTVYLLMNSLKPEDTAIYYCAAGSMVYAIMPEYYDVWGQGIQVTVSS

SEQ ID NO: 129 - protein, 123 aa, Vicugna pacos
DVQLQESGGGLVQAGGSLRLSCAPSGRTFSRNVVGWFRQAPGREREFVAHISEISGTTHYADSVKGRFTISRINAENTVYLLMNSLKPEDTAIYYCAAGSMVYAIMPEYYDVWGQGIQVTVSS

SEQ ID NO: 130 - protein, 119 aa, Vicugna pacos
QVQLQESGGGMVQPGGSLRLSCAASGRTFGIGWFRQAPGKEREFVAAIQWSGSGRTYADSVKGRFTIIRDDAKNVVYLYMDSLKPEDTAVYYCAAGRTYYSQQDSYDSWGQGTQVTVSS

SEQ ID NO: 131 - protein, 121 aa, Vicugna pacos
DVQLQESGGGLVQAGDSLRLSCKASERAFSRSYMHWFRQAPGQAREFVGRIQTNDYILYADSVRGRFIISRDYMTNTVYLQMNNLKVEDTATYYCAAEQSLMTDMEEFEFWGQGTQVVVSS

SEQ ID NO: 132 - protein, 121 aa, Vicugna pacos
DVQLQASGGGLVQAGGSLRLSCAASGAISSYHMGWLRQGPGEVRDFVATIDSSGHSIGYADSVKDRFSISRDNAKNTVYLQMNNLKPEDTAVYYCAIGRWPTVKAAFVDSWGQGTQVTVTV

SEQ ID NO: 133 - protein, 121 aa, Vicugna pacos
DVQLQESGGGLVQAGGSLRLSCAASGAISSYHMGWLRQGPGEVRDFVATIDSSGHSIGYADSVKGRFSISRDNAKNTVYLQMNNLEPEDTAVYYCAIGRWPTVKAAFVESWGQGTQVTVTD

SEQ ID NO: 134 - protein, 122 aa, Vicugna pacos
QVQLQESGGGLVQAGDSLRLSCAISGRTVSSYFMGWLRQAPPKEREFVATINWTGDNIGYADSVKGRFTISRDNSKNTVHLQMDNLKPEDTAVYYCAYGRWPTVRPESIDSWGQGTQVTVSS

SEQ ID NO: 135 - protein, 122 aa, Vicugna pacos
QVQLQESGGGLVQAGDSLRLSCAISGRTDSSYFMGWLRQAPPKEREFVATINWASDNIGYADSVKGRFTISRDNAKNTVYLQMDNLKPDDTAVYYCAYGRWPTVRPESIDSWGQGTQVTVSS

SEQ ID NO: 136 - protein, 122 aa, Vicugna pacos
QVKLQESGGGLVQAGDSLRLSCTISGRTDSSYFMGWLRQAPPKEREFVATINWDGDNIGYADSVKGRFTISRDNAKNTVHLQMDNLKPEDTAVYYCAYGRWPTVRPGSVTSWGQGTQVTVSS

SEQ ID NO: 137 - protein, 702 aa, Homo sapiens
MTGLLGLSPVSHRGVSCKYSLLFYRPLSSSCSWAQLLGNISPLHGPEPHCPADRANPVPQRGSQPPGTVAATVLLCSRFLQGFRDDGAGLRASGKDSAPTVVSGILGGSVTLPLNISVDTEIENVIWIGPKNALAFARPKENVTIMVKSYLGRLDITKWSYSLCISNLTLNDAGSYKAQINQRNFEVTTEEEFTLFVYEQLQEPQVTMKSVKVSENFSCNITLMCSVKGAEKSVLYSWTPREPHASESNGGSILTVSRTPCDPDLPYICTAQNPVSQRSSLPVHVGQFCTDPGASRGGTTGETVVGVLGEPVTLPLALPACRDTEKVVWLFNTSIISKEREEAATADPLIKSRDPYKNRVWVSSQDCSLKISQLKIEDAGPYHAYVCSEASSVTSMTHVTLLIYRRLRKPKITWSLRHSEDGICRISLTCSVEDGGNTVMYTWTPLQKEAVVSQGESHLNVSWRSSENHPNLTCTASNPVSRSSHQFLSENICSGPERNTKLWIGLFLMVCLLCVGIFSWCIWKRKGRCSVPAFCSSQAEAPADTPEPTAGHTLYSVLSQGYEKLDTPLRPARQQPTPTSDSSSDSNLTTEEDEDRPEVHKPISGRYEVFDQVTQEGAGHDPAPEGQADYDPVTPYVTEVESVVGENTMYAQVFNLQGKTPVSQKEESSATIYCSIRKPQVVPPPQQNDLEIPESPTYENFT

SEQ ID NO: 138 - DNA, 21 bp, synthetic construct
  source 1..21: mol_type = other DNA
cgcaaatgggcggtaggcgtg

SEQ ID NO: 139 - DNA, 18 bp, synthetic construct
  source 1..18: mol_type = other DNA
tagaaggcacagtcgagg

SEQ ID NO: 140 - DNA, 46 bp, synthetic construct
  source 1..46: mol_type = other DNA
tcgcggcccagccggccatggcgcaggtsmarctgcaggagtcwgg

SEQ ID NO: 141 - DNA, 52 bp, synthetic construct
  source 1..52: mol_type = other DNA
tcgcggcccagccggccatggccgatgtgcagctgcaggmgtcwggrggagg

SEQ ID NO: 142 - DNA, 51 bp, synthetic construct
  source 1..51: mol_type = other DNA
aggattgggttgtggtgcggccgctggttgtggttttggtgtcttgggttc

SEQ ID NO: 143 - DNA, 44 bp, synthetic construct
  source 1..44: mol_type = other DNA
cctgggcatttgggagcggccgcgctggggtcttcgctgtggtg